European Patent Application EP 4 365 285 A1, published May 8, 2024. Title: GLYCOSYLTRANSFERASE MUTANT, AND METHOD FOR CATALYTIC SYNTHESIS OF REBAUDIOSIDE M USING GLYCOSYLTRANSFERASE MUTANT. Applicant: XINGHUA GL STEVIA CO., LTD. The sequence listing filed with the application follows.

SEQUENCE LISTING (28 sequences)

SEQ ID NO: 1 - protein, 458 aa, synthetic construct
  REGION 1..458: note = The sequence is synthetized.
MENKTETTVRRRRRIILFPVPFQGHINPILQLANVLYSKGFSITIFHTNFNKPKTSNYPHFTFRFILDNDPQDERISNLPTHGPLAGMRIPIINEHGADELRRELELLMLASEEDEEVSCLITDALWYFAQSVADSLNLRRLVLMTSSLFNFHAHVSLPQFDELGYLDPDDKTRLEEQASGFPMLKVKDIKSAYSNWQILKEILGKMIKQTKASSGVIWNSFKELEESELETVIREIPAPSFLIPLPKHLTASSSSLLDHDRTVFQWLDQQPPSSVLYVSFGSTSEVDEKDFLEIARGLVDSKQSFLWVVRPGFVKGSTWVEPLPDGFLGERGRIVKWVPQQEVLAHGAIGAFWTHSGWNSTLESVCEGVPMIFSDFGLDQPLNARYMSDVLKVGVYLENGWERGEIANAIRRVMVDEEGEYIRQNARVLKQKADVSLMKGGSSYESLESLVSYISSL

SEQ ID NO: 2 - DNA, 1377 bp, synthetic construct
  misc_feature 1..1377: note = The sequence is synthetized.
  source 1..1377: mol_type = other DNA
atggaaaataaaaccgaaaccaccgtccgccgtcgtcgccgtatcattctgttcccggtcccgttccagggccacatcaacccgattctgcaactggcgaacgtgctgtattcgaaaggtttcagcatcaccatcttccatacgaacttcaacaagccgaagaccagcaattacccgcactttacgttccgttttattctggataacgacccgcaggatgaacgcatctctaatctgccgacccacggcccgctggcgggtatgcgtattccgattatcaacgaacacggcgcagatgaactgcgtcgcgaactggaactgctgatgctggccagcgaagaagatgaagaagtttcttgcctgatcaccgacgcactgtggtattttgcccagtctgttgcagatagtctgaacctgcgtcgcctggtcctgatgaccagcagcctgttcaattttcatgcccacgttagtctgccgcagttcgatgaactgggttatctggacccggatgacaaaacccgcctggaagaacaggcgagcggctttccgatgctgaaagtcaaggatattaagtcagcgtactcgaactggcagattctgaaagaaatcctgggtaaaatgattaagcaaaccaaagcaagttccggcgtcatctggaatagtttcaaagaactggaagaatccgaactggaaacggtgattcgtgaaatcccggctccgagttttctgattccgctgccgaagcatctgaccgcgagcagcagcagcctgctggatcacgaccgcacggtgtttcagtggctggatcagcaaccgccgagttccgtgctgtatgttagcttcggtagtacctcggaagtggatgaaaaggactttctggaaatcgctcgtggcctggttgatagcaaacaatctttcctgtgggtggttcgcccgggttttgtgaagggctctacgtgggttgaaccgctgccggacggcttcctgggtgaacgtggccgcattgtcaaatgggtgccgcagcaagaagtgctggcgcatggcgcgattggcgcgttttggacccactccggttggaactcaacgctggaatcggtttgtgaaggtgtcccgatgattttctcagattttggcctggaccagccgctgaatgcacgttatatgtcggatgttctgaaagtcggtgtgtacctggaaaacggttgggaacgcggcgaaattgcgaatgccatccgtcgcgttatggtcgatgaagaaggcgaatacattcgtcagaatgctcgcgtcctgaaacaaaaggcggacgtgagcctgatgaaaggcggttcatcgtatgaaagtctggaatccctggtttcatacatcagctctctgtaa

SEQ ID NO: 3 - DNA, 1377 bp, synthetic construct
  misc_feature 1..1377: note = The sequence is synthetized.
  source 1..1377: mol_type = other DNA
atggaaaataaaaccgaaaccaccgtccgccgtcgtcgccgtatcattctgttcccggtcccgttccagggccacatcaacccgattctgcaactggcgaacgtgctgtattcgaaaggtttcagcatcaccatcttccatacgaacttcaacaagccgaagaccagcaattacccgcactttacgttccgttttattctggataacgacccgcaggatgaacgcatctctaatctgccgacccacggcccgctggcggacatgcgtattccgattatcaacgaacacggcgcagatgaactgcgtcgcgaactggaactgctgatgctggccagcgaagaagatgaagaagtttcttgcctgatcaccgacgcactgtggtattttgcccagtctgttgcagatagtctgaacctgcgtcgcctggtcctgatgaccagcagcctgttcaattttcatgcccacgttagtctgccgcagttcgatgaactgggttatctggacccggatgacaaaacccgcctggaagaacaggcgagcggctttccgatgctgaaagtcaaggatattaagtcagcgtactcgaactggcagattctgaaagaaatcctgggtaaaatgattaagcaaaccaaagcaagttccggcgtcatctggaatagtttcaaagaactggaagaatccgaactggaaacggtgattcgtgaaatcccggctccgagttttctgattccgctgccgaagcatctgaccgcgagcagcagcagcctgctggatcacgaccgcacggtgtttcagtggctggatcagcaaccgccgagttccgtgctgtatgttagcttcggtagtacctcggaagtggatgaaaaggactttctggaaatcgctcgtggcctggttgatagcaaacaatctttcctgtgggtggttcgcccgggttttgtgaagggctctacgtgggttgaaccgctgccggacggcttcctgggtgaacgtggccgcattgtcaaatgggtgccgcagcaagaagtgctggcgcatggcgcgattggcgcgttttggacccactccggttggaactcaacgctggaatcggtttgtgaaggtgtcccgatgattttctcagattttggcctggaccagccgctgaatgcacgttatatgtcggatgttctgaaagtcggtgtgtacctggaaaacggttgggaacgcggcgaaattgcgaatgccatccgtcgcgttatggtcgatgaagaaggcgaatacattcgtcagaatgctcgcgtcctgaaacaaaaggcggacgtgagcctgatgaaaggcggttcatcgtatgaaagtctggaatccctggtttcatacatcagctctctgtaa

SEQ ID NO: 4 - DNA, 1377 bp, synthetic construct
  misc_feature 1..1377: note = The sequence is synthetized.
  source 1..1377: mol_type = other DNA
atggaaaataaaaccgaaaccaccgtccgccgtcgtcgccgtatcattctgttcccggtcccgttccagggccacatcaacccgattctgcaactggcgaacgtgctgtattcgaaaggtttcagcatcaccatcttccatacgaacttcaacaagccgaagaccagcaattacccgcactttacgttccgttttattctggataacgacccgcaggatgaacgcatctctaatctgccgacccacggcccgctggcgggtatgcgtattccgattatcaacgaacacggcgcagatgaactgcgtcgcgaactggaactgctgatgctggccagcgaagaagatgaagaagtttcttgcctgatcaccgacgcactgtggtattttgcccagtctgttgcagatagtctgaacctgcgtcgcctggtcctgatgaccgacagcctgttcaattttcatgcccacgttagtctgccgcagttcgatgaactgggttatctggacccggatgacaaaacccgcctggaagaacaggcgagcggctttccgatgctgaaagtcaaggatattaagtcagcgtactcgaactggcagattctgaaagaaatcctgggtaaaatgattaagcaaaccaaagcaagttccggcgtcatctggaatagtttcaaagaactggaagaatccgaactggaaacggtgattcgtgaaatcccggctccgagttttctgattccgctgccgaagcatctgaccgcgagcagcagcagcctgctggatcacgaccgcacggtgtttcagtggctggatcagcaaccgccgagttccgtgctgtatgttagcttcggtagtacctcggaagtggatgaaaaggactttctggaaatcgctcgtggcctggttgatagcaaacaatctttcctgtgggtggttcgcccgggttttgtgaagggctctacgtgggttgaaccgctgccggacggcttcctgggtgaacgtggccgcattgtcaaatgggtgccgcagcaagaagtgctggcgcatggcgcgattggcgcgttttggacccactccggttggaactcaacgctggaatcggtttgtgaaggtgtcccgatgattttctcagattttggcctggaccagccgctgaatgcacgttatatgtcggatgttctgaaagtcggtgtgtacctggaaaacggttgggaacgcggcgaaattgcgaatgccatccgtcgcgttatggtcgatgaagaaggcgaatacattcgtcagaatgctcgcgtcctgaaacaaaaggcggacgtgagcctgatgaaaggcggttcatcgtatgaaagtctggaatccctggtttcatacatcagctctctgtaa

SEQ ID NO: 5 - DNA, 1377 bp, synthetic construct
  misc_feature 1..1377: note = The sequence is synthetized.
  source 1..1377: mol_type = other DNA
atggaaaataaaaccgaaaccaccgtccgccgtcgtcgccgtatcattctgttcccggtcccgttccagggccacatcaacccgattctgcaactggcgaacgtgctgtattcgaaaggtttcagcatcaccatcttccatacgaacttcaacaagccgaagaccagcaattacccgcactttacgttccgttttattctggataacgacccgcaggatgaacgcatctctaatctgccgacccacggcccgctggcgggtatgcgtattccgattatcaacgaacacggcgcagatgaactgcgtcgcgaactggaactgctgatgctggccagcgaagaagatgaagaagtttcttgcctgatcaccgacgcactgtggtattttgcccagtctgttgcagatagtctgaacctgcgtcgcctggtcctgatgaccaacagcctgttcaattttcatgcccacgttagtctgccgcagttcgatgaactgggttatctggacccggatgacaaaacccgcctggaagaacaggcgagcggctttccgatgctgaaagtcaaggatattaagtcagcgtactcgaactggcagattctgaaagaaatcctgggtaaaatgattaagcaaaccaaagcaagttccggcgtcatctggaatagtttcaaagaactggaagaatccgaactggaaacggtgattcgtgaaatcccggctccgagttttctgattccgctgccgaagcatctgaccgcgagcagcagcagcctgctggatcacgaccgcacggtgtttcagtggctggatcagcaaccgccgagttccgtgctgtatgttagcttcggtagtacctcggaagtggatgaaaaggactttctggaaatcgctcgtggcctggttgatagcaaacaatctttcctgtgggtggttcgcccgggttttgtgaagggctctacgtgggttgaaccgctgccggacggcttcctgggtgaacgtggccgcattgtcaaatgggtgccgcagcaagaagtgctggcgcatggcgcgattggcgcgttttggacccactccggttggaactcaacgctggaatcggtttgtgaaggtgtcccgatgattttctcagattttggcctggaccagccgctgaatgcacgttatatgtcggatgttctgaaagtcggtgtgtacctggaaaacggttgggaacgcggcgaaattgcgaatgccatccgtcgcgttatggtcgatgaagaaggcgaatacattcgtcagaatgctcgcgtcctgaaacaaaaggcggacgtgagcctgatgaaaggcggttcatcgtatgaaagtctggaatccctggtttcatacatcagctctctgtaa

SEQ ID NO: 6 - DNA, 1377 bp, synthetic construct
  misc_feature 1..1377: note = The sequence is synthetized.
  source 1..1377: mol_type = other DNA
atggaaaataaaaccgaaaccaccgtccgccgtcgtcgccgtatcattctgttcccggtcccgttccagggccacatcaacccgattctgcaactggcgaacgtgctgtattcgaaaggtttcagcatcaccatcttccatacgaacttcaacaagccgaagaccagcaattacccgcactttacgttccgttttattctggataacgacccgcaggatgaacgcatctctaatctgccgacccacggcccgctggcgggtatgcgtattccgattatcaacgaacacggcgcagatgaactgcgtcgcgaactggaactgctgatgctggccagcgaagaagatgaagaagtttcttgcctgatcaccgacgcactgtggtattttgcccagtctgttgcagatagtctgaacctgcgtcgcctggtcctgatgaccagcagcctgttcaattttcatgcccacgttagtctgccgcagttcgatgaactgggttatctggacccggatgacaaaacccgcctggaagaacaggcgagcggctttccgatgctgaaagtcaaggatattaagtcagcgtaccaaaactggcagattctgaaagaaatcctgggtaaaatgattaagcaaaccaaagcaagttccggcgtcatctggaatagtttcaaagaactggaagaatccgaactggaaacggtgattcgtgaaatcccggctccgagttttctgattccgctgccgaagcatctgaccgcgagcagcagcagcctgctggatcacgaccgcacggtgtttcagtggctggatcagcaaccgccgagttccgtgctgtatgttagcttcggtagtacctcggaagtggatgaaaaggactttctggaaatcgctcgtggcctggttgatagcaaacaatctttcctgtgggtggttcgcccgggttttgtgaagggctctacgtgggttgaaccgctgccggacggcttcctgggtgaacgtggccgcattgtcaaatgggtgccgcagcaagaagtgctggcgcatggcgcgattggcgcgttttggacccactccggttggaactcaacgctggaatcggtttgtgaaggtgtcccgatgattttctcagattttggcctggaccagccgctgaatgcacgttatatgtcggatgttctgaaagtcggtgtgtacctggaaaacggttgggaacgcggcgaaattgcgaatgccatccgtcgcgttatggtcgatgaagaaggcgaatacattcgtcagaatgctcgcgtcctgaaacaaaaggcggacgtgagcctgatgaaaggcggttcatcgtatgaaagtctggaatccctggtttcatacatcagctctctgtaa

SEQ ID NO: 7 - DNA, 1377 bp, synthetic construct
  misc_feature 1..1377: note = The sequence is synthetized.
  source 1..1377: mol_type = other DNA
atggaaaataaaaccgaaaccaccgtccgccgtcgtcgccgtatcattctgttcccggtcccgttccagggccacatcaacccgattctgcaactggcgaacgtgctgtattcgaaaggtttcagcatcaccatcttccatacgaacttcaacaagccgaagaccagcaattacccgcactttacgttccgttttattctggataacgacccgcaggatgaacgcatctctaatctgccgacccacggcccgctggcgggtatgcgtattccgattatcaacgaacacggcgcagatgaactgcgtcgcgaactggaactgctgatgctggccagcgaagaagatgaagaagtttcttgcctgatcaccgacgcactgtggtattttgcccagtctgttgcagatagtctgaacctgcgtcgcctggtcctgatgaccagcagcctgttcaattttcatgcccacgttagtctgccgcagttcgatgaactgggttatctggacccggatgacaaaacccgcctggaagaacaggcgagcggctttccgatgctgaaagtcaaggatattaagtcagcgtactcgaactggcagatttacaaagaaatcctgggtaaaatgattaagcaaaccaaagcaagttccggcgtcatctggaatagtttcaaagaactggaagaatccgaactggaaacggtgattcgtgaaatcccggctccgagttttctgattccgctgccgaagcatctgaccgcgagcagcagcagcctgctggatcacgaccgcacggtgtttcagtggctggatcagcaaccgccgagttccgtgctgtatgttagcttcggtagtacctcggaagtggatgaaaaggactttctggaaatcgctcgtggcctggttgatagcaaacaatctttcctgtgggtggttcgcccgggttttgtgaagggctctacgtgggttgaaccgctgccggacggcttcctgggtgaacgtggccgcattgtcaaatgggtgccgcagcaagaagtgctggcgcatggcgcgattggcgcgttttggacccactccggttggaactcaacgctggaatcggtttgtgaaggtgtcccgatgattttctcagattttggcctggaccagccgctgaatgcacgttatatgtcggatgttctgaaagtcggtgtgtacctggaaaacggttgggaacgcggcgaaattgcgaatgccatccgtcgcgttatggtcgatgaagaaggcgaatacattcgtcagaatgctcgcgtcctgaaacaaaaggcggacgtgagcctgatgaaaggcggttcatcgtatgaaagtctggaatccctggtttcatacatcagctctctgtaa

SEQ ID NO: 8 - DNA, 1377 bp, synthetic construct
  misc_feature 1..1377: note = The sequence is synthetized.
  source 1..1377: mol_type = other DNA
atggaaaataaaaccgaaaccaccgtccgccgtcgtcgccgtatcattctgttcccggtcccgttccagggccacatcaacccgattctgcaactggcgaacgtgctgtattcgaaaggtttcagcatcaccatcttccatacgaacttcaacaagccgaagaccagcaattacccgcactttacgttccgttttattctggataacgacccgcaggatgaacgcatctctaatctgccgacccacggcccgctggcgggtatgcgtattccgattatcaacgaacacggcgcagatgaactgcgtcgcgaactggaactgctgatgctggccagcgaagaagatgaagaagtttcttgcctgatcaccgacgcactgtggtattttgcccagtctgttgcagatagtctgaacctgcgtcgcctggtcctgatgaccagcagcctgttcaattttcatgcccacgttagtctgccgcagttcgatgaactgggttatctggacccggatgacaaaacccgcctggaagaacaggcgagcggctttccgatgctgaaagtcaaggatattaagtcagcgtactcgaactggcagattctgaaagaaatcctgggtaaaatgattaagcaaaccaaagcaagttccggcgtcatctggaatagtttcaaagaactggaagaatccgaactggaaacggtgattcgtgaaatcccggctccgagttttctgattccgctgccgaagcatctgaccgcgagcagcagcagcctgctggatcacgaccgcacggtgtttcagtggctggatcagcaaccgccgagttccgtgctgtatgttagcttcggtagtagctcggaagtggatgaaaaggactttctggaaatcgctcgtggcctggttgatagcaaacaatctttcctgtgggtggttcgcccgggttttgtgaagggctctacgtgggttgaaccgctgccggacggcttcctgggtgaacgtggccgcattgtcaaatgggtgccgcagcaagaagtgctggcgcatggcgcgattggcgcgttttggacccactccggttggaactcaacgctggaatcggtttgtgaaggtgtcccgatgattttctcagattttggcctggaccagccgctgaatgcacgttatatgtcggatgttctgaaagtcggtgtgtacctggaaaacggttgggaacgcggcgaaattgcgaatgccatccgtcgcgttatggtcgatgaagaaggcgaatacattcgtcagaatgctcgcgtcctgaaacaaaaggcggacgtgagcctgatgaaaggcggttcatcgtatgaaagtctggaatccctggtttcatacatcagctctctgtaa

SEQ ID NO: 9 - DNA, 1377 bp, synthetic construct
  misc_feature 1..1377: note = The sequence is synthetized.
  source 1..1377: mol_type = other DNA
atggaaaataaaaccgaaaccaccgtccgccgtcgtcgccgtatcattctgttcccggtcccgttccagggccacatcaacccgattctgcaactggcgaacgtgctgtattcgaaaggtttcagcatcaccatcttccatacgaacttcaacaagccgaagaccagcaattacccgcactttacgttccgttttattctggataacgacccgcaggatgaacgcatctctaatctgccgacccacggcccgctggcgggtatgcgtattccgattatcaacgaacacggcgcagatgaactgcgtcgcgaactggaactgctgatgctggccagcgaagaagatgaagaagtttcttgcctgatcaccgacgcactgtggtattttgcccagtctgttgcagatagtctgaacctgcgtcgcctggtcctgatgaccagcagcctgttcaattttcatgcccacgttagtctgccgcagttcgatgaactgggttatctggacccggatgacaaaacccgcctggaagaacaggcgagcggctttccgatgctgaaagtcaaggatattaagtcagcgtactcgaactggcagattctgaaagaaatcctgggtaaaatgattaagcaaaccaaagcaagttccggcgtcatctggaatagtttcaaagaactggaagaatccgaactggaaacggtgattcgtgaaatcccggctccgagttttctgattccgctgccgaagcatctgaccgcgagcagcagcagcctgctggatcacgaccgcacggtgtttcagtggctggatcagcaaccgccgagttccgtgctgtatgttagcttcggtagtacctgggaagtggatgaaaaggactttctggaaatcgctcgtggcctggttgatagcaaacaatctttcctgtgggtggttcgcccgggttttgtgaagggctctacgtgggttgaaccgctgccggacggcttcctgggtgaacgtggccgcattgtcaaatgggtgccgcagcaagaagtgctggcgcatggcgcgattggcgcgttttggacccactccggttggaactcaacgctggaatcggtttgtgaaggtgtcccgatgattttctcagattttggcctggaccagccgctgaatgcacgttatatgtcggatgttctgaaagtcggtgtgtacctggaaaacggttgggaacgcggcgaaattgcgaatgccatccgtcgcgttatggtcgatgaagaaggcgaatacattcgtcagaatgctcgcgtcctgaaacaaaaggcggacgtgagcctgatgaaaggcggttcatcgtatgaaagtctggaatccctggtttcatacatcagctctctgtaa

SEQ ID NO: 10 - DNA, 1377 bp, synthetic construct
  misc_feature 1..1377: note = The sequence is synthetized.
  source 1..1377: mol_type = other DNA
atggaaaataaaaccgaaaccaccgtccgccgtcgtcgccgtatcattctgttcccggtcccgttccagggccacatcaacccgattctgcaactggcgaacgtgctgtattcgaaaggtttcagcatcaccatcttccatacgaacttcaacaagccgaagaccagcaattacccgcactttacgttccgttttattctggataacgacccgcaggatgaacgcatctctaatctgccgacccacggcccgctggcgggtatgcgtattccgattatcaacgaacacggcgcagatgaactgcgtcgcgaactggaactgctgatgctggccagcgaagaagatgaagaagtttcttgcctgatcaccgacgcactgtggtattttgcccagtctgttgcagatagtctgaacctgcgtcgcctggtcctgatgaccagcagcctgttcaattttcatgcccacgttagtctgccgcagttcgatgaactgggttatctggacccggatgacaaaacccgcctggaagaacaggcgagcggctttccgatgctgaaagtcaaggatattaagtcagcgtactcgaactggcagattctgaaagaaatcctgggtaaaatgattaagcaaaccaaagcaagttccggcgtcatctggaatagtttcaaagaactggaagaatccgaactggaaacggtgattcgtgaaatcccggctccgagttttctgattccgctgccgaagcatctgaccgcgagcagcagcagcctgctggatcacgaccgcacggtgtttcagtggctggatcagcaaccgccgagttccgtgctgtatgttagcttcggtagtacctcggaagtggatgaaaaggactttctggaaatcgctcgtggcctggttgatagcaaacaatctttcctgtgggtggttcgcccgggttttgtgaagggctctacgtgggttgaaccgctgccggacggcttcctgggtgaacgtggccgcattgtcaaatgggtgccgcagcaagaagtgctggcgcatggcgcgattggcgcgttttggacccactccggttggaactcaacgctggaatcggtttgtgaaggtgtcccgatgattttctcagattttccactggaccagccgctgaatgcacgttatatgtcggatgttctgaaagtcggtgtgtacctggaaaacggttgggaacgcggcgaaattgcgaatgccatccgtcgcgttatggtcgatgaagaaggcgaatacattcgtcagaatgctcgcgtcctgaaacaaaaggcggacgtgagcctgatgaaaggcggttcatcgtatgaaagtctggaatccctggtttcatacatcagctctctgtaa

SEQ ID NO: 11 - DNA, 2418 bp, synthetic construct
  misc_feature 1..2418: note = The sequence is synthetized.
  source 1..2418: mol_type = other DNA
atggccgaacgtgtcctgacccgtgtccatagtctgcgtgaacgtgttgatgctaccctggctgcccaccgtaatgaaatcctgctgtttctgagtcgtattgaaagccacggcaaaggtatcctgaaaccgcacgaactgctggcagaatttgatgctattcgccaggatgacaaaaacaaactgaacgaacatgcattcgaagaactgctgaaaagcacccaagaagctatcgtcctgccgccgtgggtggcactggcaattcgtctgcgcccgggcgtttgggaatacatccgtgttaacgtcaatgcgctggttgtggaagaactgagtgtgccggaatatctgcagtttaaagaagaactggtcgatggcgcgtccaacggtaatttcgtgctggaactggactttgaaccgttcaccgcctcatttccgaaaccgaccctgacgaaatcgattggcaacggtgttgaatttctgaatcgtcatctgagcgccaaaatgttccacgataaagaatctatgaccccgctgctggaatttctgcgcgcacatcactataaaggtaaaaccatgatgctgaacgatcgtattcagaacagcaatacgctgcaaaatgtgctgcgcaaagcggaagaatacctgatcatgctgccgccggaaaccccgtacttcgaatttgaacataaattccaggaaattggcctggaaaaaggctggggtgatacggcagaacgtgtgctggaaatggtttgcatgctgctggatctgctggaagctccggacagctgtaccctggaaaaatttctgggtcgcattccgatggttttcaacgtcgtgatcctgtctccgcacggctattttgcgcaggaaaatgtcctgggttacccggataccggcggtcaggttgtctatattctggaccaagtgccggccctggaacgtgaaatgctgaaacgcatcaaagaacagggcctggatattatcccgcgtattctgatcgtcacccgtctgctgccggacgcagtgggcaccacgtgcggtcaacgtattgaaaaagtgtatggcgctgaacattcacacatcctgcgtgttccgtttcgcaccgaaaaaggtattgtccgtaaatggatctcgcgctttgaagtgtggccgtacatggaaacgttcattgaagatgttgcaaaagaaatctcagcggaactgcaggccaaaccggacctgattatcggcaactatagcgaaggtaatctggcggcctctctgctggcccataaactgggcgtgacccaatgtacgattgcacacgctctggaaaaaaccaaatatccggattcggacatctactggaaaaaattcgatgaaaaataccatttcagctctcagttcaccgcagatctgattgctatgaaccacacggactttattatcaccagtacgttccaggaaatcgcgggctccaaagataccgtgggtcaatacgaaagtcatatggcctttacgatgccgggcctgtatcgcgtggttcacggtatcaacgttttcgatccgaaattcaacattgtctccccgggtgcagacatcaatctgtatttttcatactcggaaaccgaaaaacgtctgacggctttccatccggaaatcgatgaactgctgtatagcgatgtggaaaacgacgaacacctgtgcgttctgaaagatcgcaccaaaccgattctgtttacgatggcgcgtctggaccgcgttaaaaatctgaccggcctggtcgaatggtacgccaaaaacccgcgtctgcgcggtctggtgaatctggtcgtggttggcggtgatcgtcgcaaagaatctaaagacctggaagaacaggcggaaatgaagaaaatgtacgaactgatcgaaacccataacctgaatggccagttccgttggatcagttcccaaatgaaccgtgttcgcaatggcgaactgtatcgctacatcgcagatacgaaaggtgcttttgtccagccggcgttttacgaagccttcggcctgaccgtcgtggaagcgatgacgtgcggtctgccgaccttcgcaacgaatcatggcggcccggcagaaattatcgttcacggcaaaagtggttttcatattgatccgtatcacggcgaacaggcagctgatctgctggccgactttttcgaaaaatgtaaaaaagacccgtcacattgggaaaccatttcgatgggcggtctgaaacgcatcgaagaaaaatatacctggcaaatttacagcgaatctctgctgacgctggcggccgtgtacggtttctggaaacacgtttctaaactggatcgtctggaaattcgtcgctatctggaaatgttttatgcgctgaaataccgcaaaatggcggaagccgtgccgctggcagctgaataa

SEQ ID NO: 12 - DNA, 2595 bp, synthetic construct
  misc_feature 1..2595: note = The sequence is synthetized.
  source 1..2595: mol_type = other DNA
atgagcgcaggagctgattctccctcaagtcaacccttcttggctagcccgcgtggtgttatcaccccgcgtaccttcacccgctcgctgtcgttcgcaggcggtacgccgtccgaaattttgaaggcgggcttggttcacagccgtaatgagctggtgctgctgttcagccgttgcatggcaaagagcaaagcggacaagccaattctgttaccgcatattattatggatgagttatgcgccgtgtgtgatgaatgcaataatccgatgctgaaatctggtgagatcgcggcgatcttgaaaaccgttcaggaagcggtagttatcgcaccgcgaatcgccttcgcgttgagacctacgatgggtgaatggtactacgttcgcgtgtctgttgaagatatgcgcgttgaagaaatgaccgctgcgcactatctcgcgtttaaagagaagctggttccactggaccaagatcgtcacggctacgacccattcgtgctggagctggacttgaagccgtttggcgcacaccagcctaagattagcctgcaaagccacatcggtaacggtgttagcttcctgaatcgcacgctgtcggcgaaaatgttttcccagaacgccaatgcggaaggcagccaattgatgttggacttcctgcgtgaatttaagcacggaggcgaaaagttactgctaagcccgcgtgtgaatagcgtgcagaaattgcgccactcactgctgcgtgctgaccgcttactggagaagcacgaagacgaggacccgctgtctgttgtgcaaggtatcgacgagctgggcttcctgccgggttggggtaacactgttggccgtgttagagagtcctttcagctgctgttggacatcatccaggcaccagacgctgatactctggaaaagttcctggcccgcttgccgctgatggttaaagttgtcatcttgtcgccgcatggttatttcggtcaaaccaatgtgttgggtatgccggacaccggtggtcaggtggtctacattctggaccaggttcgtgcgatggagcgtgagatgcagcagcgtctagatgaagcgggccttcagaatgtgaaagcggatgttgttgtgctgacccgtctgattccggatgcacatggtacttcctgcaacgagcgcttggagccgattagtggctgccaaaacgcgcgtatcctgcgtgttccgtttcgggatagcgaaggtcgtatcctgaatcattgggtttccaggttcgatctgtggccgtatctggagcgctttaccattgacgccacgaaggaaatcctggctgaaatgggcggtaaaccggacttcattatcggcaactatagcgatggtaacttagtggcgaccctcatgagccatcgtatgaacgtgacccagtgtaacattgcgcatgcgctggaaaaaaccaaatacgatgatgccgacatttactggcagaagcttgaagacaaataccattttagctgccaatttacggccgacctgatcgcaatgaactctgcggattttatcgtcacctccacctaccaggagatcgctggtcatgaggaaatggtgggccaatatgagagctataagagctttaccatgccacagctgtaccgcgttgtggagggcattgacatctacaacccgaagttcaacattgtgagcccgggtgcggacctggacatctactttccgtaccaggagaaggagaggcgtttgaccggcctgcataaggacattgaagcgctgctgtttgacccggattttaaaggtacggtcggtcagttagaggacagagacaaaccgatcctgttttctatggcgcgtttggacaaagtgaagaacctgactggcctggccgagtggtacgcgggcaatcagcgtttgcgtggtctggtcaacctggtcatagtcggtggcgttattgatccggctgctacgatggaccgcgaagaggcagcggagtgcgaacacatgcacgaacttgtcgagaagtataaaatgcatggcacgttccgctggattgttgctcagaagaaccgtgtacgtaacggcgagctgtatagatacatcgctgatactcgtggtgctttcgcccaaccggcactgtacgaagcctttgggctgaccgtgatcgaggcgatgacctgtggtcttccgaccttcgcaaccaaccacggcggtccgtccgaaatcattaaacacaagaaaagcggcttccatatcgacccgtatcacggtgcggaagcggcggatctgatggcggatttctttgaacgttctcaaaaggagccgtctcattggaccaagatctccgaggcggcgcaagaacgtatttttagccgttacacgtggtcaatctacgcaaagcgcctggtgaccttgagccacgtgtataccttctggaaacacgtgaccagcctggagagccgcgaaaccaaacgttatctggagatgttctatattctgcaaatgcgtaaattggtagccaaaatgtcggaagagaccgtggaaaaggagaaggcggcggcagaggcaggtccggcgggcccgcctaaagttggctttggtgctatgtaa

SEQ ID NO: 13 - DNA, 36 bp, synthetic construct
  misc_feature 1..36: note = The sequence is synthetized.
  source 1..36: mol_type = other DNA
ccgctggcggacatgcgtattccgattatcaacgaa

SEQ ID NO: 14 - DNA, 36 bp, synthetic construct
  misc_feature 1..36: note = The sequence is synthetized.
  source 1..36: mol_type = other DNA
aatacgcatgtccgccagcgggccgtgggtcggcag

SEQ ID NO: 15 - DNA, 36 bp, synthetic construct
  misc_feature 1..36: note = The sequence is synthetized.
  source 1..36: mol_type = other DNA
ctgatgaccgacagcctgttcaattttcatgcccac

SEQ ID NO: 16 - DNA, 36 bp, synthetic construct
  misc_feature 1..36: note = The sequence is synthetized.
  source 1..36: mol_type = other DNA
gaacaggctgtcggtcatcaggaccaggcgacgcag

SEQ ID NO: 17 - DNA, 36 bp, synthetic construct
  misc_feature 1..36: note = The sequence is synthetized.
  source 1..36: mol_type = other DNA
ctgatgaccaacagcctgttcaattttcatgcccac

SEQ ID NO: 18 - DNA, 36 bp, synthetic construct
  misc_feature 1..36: note = The sequence is synthetized.
  source 1..36: mol_type = other DNA
gaacaggctgttggtcatcaggaccaggcgacgcag

SEQ ID NO: 19 - DNA, 36 bp, synthetic construct
  misc_feature 1..36: note = The sequence is synthetized.
  source 1..36: mol_type = other DNA
tcagcgtaccaaaactggcagattctgaaagaaatc

SEQ ID NO: 20 - DNA, 36 bp, synthetic construct
  misc_feature 1..36: note = The sequence is synthetized.
  source 1..36: mol_type = other DNA
ctgccagttttggtacgctgacttaatatccttgac

SEQ ID NO: 21 - DNA, 36 bp, synthetic construct
  misc_feature 1..36: note = The sequence is synthetized.
  source 1..36: mol_type = other DNA
tggcagatttacaaagaaatcctgggtaaaatgatt

SEQ ID NO: 22 - DNA, 36 bp, synthetic construct
  misc_feature 1..36: note = The sequence is synthetized.
  source 1..36: mol_type = other DNA
gatttctttgtaaatctgccagttcgagtacgctga

SEQ ID NO: 23 - DNA, 36 bp, synthetic construct
  misc_feature 1..36: note = The sequence is synthetized.
  source 1..36: mol_type = other DNA
ttcggtagtagctcggaagtggatgaaaaggacttt

SEQ ID NO: 24 - DNA, 36 bp, synthetic construct
  misc_feature 1..36: note = The sequence is synthetized.
  source 1..36: mol_type = other DNA
cacttccgagctactaccgaagctaacatacagcac

SEQ ID NO: 25 - DNA, 36 bp, synthetic construct
  misc_feature 1..36: note = The sequence is synthetized.
  source 1..36: mol_type = other DNA
ggtagtacctgggaagtggatgaaaaggactttctg

SEQ ID NO: 26 - DNA, 36 bp, synthetic construct
  misc_feature 1..36: note = The sequence is synthetized.
  source 1..36: mol_type = other DNA
atccacttcccaggtactaccgaagctaacatacag

SEQ ID NO: 27 - DNA, 36 bp, synthetic construct
  misc_feature 1..36: note = The sequence is synthetized.
  source 1..36: mol_type = other DNA
tcagattttccactggaccagccgctgaatgcacgt

SEQ ID NO: 28 - DNA, 36 bp, synthetic construct
  misc_feature 1..36: note = The sequence is synthetized.
  source 1..36: mol_type = other DNA
ctggtccagtggaaaatctgagaaaatcatcgggac